European Patent Specification EP 3 861 139 B1, published August 7, 2024. Title: IDENTIFICAZIONE DI BIOMARCATORI MOLECOLARI PREDITTIVI DI RISPOSTA AL TRATTAMENTO RADIOCHEMOTERAPICO NEL CARCINOMA DELLA CERVICE. Applicant: Università Cattolica del Sacro Cuore [UCSC] Agenzia nazionale per le nuove tecnologie, l'energia e lo sviluppo economico sostenibile (E. The sequence listing filed with the application follows.

SEQUENCE LISTING (62 sequences)

SEQ ID NO: 1 - DNA, 19 bp, Artificial Sequence
  >Homo sapiens
ccaaccgcgagaagatgac

SEQ ID NO: 2 - DNA, 20 bp, Artificial Sequence
  >Homo sapiens
tagcacagcctggatagcaa

SEQ ID NO: 3 - DNA, 20 bp, Artificial Sequence
  >Homo sapiens
agcagagcaaactcctctca

SEQ ID NO: 4 - DNA, 22 bp, Artificial Sequence
  >Homo sapiens
ttcactactccaggaggaaacc

SEQ ID NO: 5 - DNA, 22 bp, Artificial Sequence
  >Homo sapiens
cctggaaaatgctttcctgaac

SEQ ID NO: 6 - DNA, 20 bp, Artificial Sequence
  >Homo sapiens
tggagtcatacagccgatca

SEQ ID NO: 7 - DNA, 21 bp, Artificial Sequence
  >Homo sapiens
cctgaagtgggatgacccata

SEQ ID NO: 8 - DNA, 20 bp, Artificial Sequence
  >Homo sapiens
tcttccgcccatacttgtca

SEQ ID NO: 9 - DNA, 19 bp, Artificial Sequence
  >Homo sapiens
ttagctgtgctcgcgctac

SEQ ID NO: 10 - DNA, 22 bp, Artificial Sequence
  >Homo sapiens
ctctgctggatgacgtgagtaa

SEQ ID NO: 11 - DNA, 21 bp, Artificial Sequence
  >Homo sapiens
ctgcatacgagcgtttccaaa

SEQ ID NO: 12 - DNA, 22 bp, Artificial Sequence
  >Homo sapiens
ggcttgggtccaaatactcaac

SEQ ID NO: 13 - DNA, 22 bp, Artificial Sequence
  >Homo sapiens
gttctacggtgacgaggagaaa

SEQ ID NO: 14 - DNA, 20 bp, Artificial Sequence
  >Homo sapiens
aaactggccgacagagcata

SEQ ID NO: 15 - DNA, 20 bp, Artificial Sequence
  >Homo sapiens
cgagctaagcccaaggtgta

SEQ ID NO: 16 - DNA, 24 bp, Artificial Sequence
  >Homo sapiens
tctcatctccacctactgtttcac

SEQ ID NO: 17 - DNA, 20 bp, Artificial Sequence
  >Homo sapiens
tgccgaacatgactcctgaa

SEQ ID NO: 18 - DNA, 19 bp, Artificial Sequence
  >Homo sapiens
attggggctgcgtagttca

SEQ ID NO: 19 - DNA, 21 bp, Artificial Sequence
  >Homo sapiens
agaatggatgctcagctgtca

SEQ ID NO: 20 - DNA, 22 bp, Artificial Sequence
  >Homo sapiens
gttacactcctggacctggaaa

SEQ ID NO: 21 - DNA, 21 bp, Artificial Sequence
  >Homo sapiens
gaacgggaagcttgtcatcaa

SEQ ID NO: 22 - DNA, 20 bp, Artificial Sequence
  >Homo sapiens
atcgccccacttgattttgg

SEQ ID NO: 23 - DNA, 20 bp, Artificial Sequence
  >Homo sapiens
aagacctggcaacggatgac

SEQ ID NO: 24 - DNA, 24 bp, Artificial Sequence
  >Homo sapiens
ttgagaatcctttccaacccagac

SEQ ID NO: 25 - DNA, 21 bp, Artificial Sequence
  >Homo sapiens
tgtacggcttagaggacttcc

SEQ ID NO: 26 - DNA, 20 bp, Artificial Sequence
  >Homo sapiens
tcccatttggcacgatttcc

SEQ ID NO: 27 - DNA, 21 bp, Artificial Sequence
  >Homo sapiens
cgctatagccgtttgagggaa

SEQ ID NO: 28 - DNA, 20 bp, Artificial Sequence
  >Homo sapiens
ggcaagtttggctcaatgca

SEQ ID NO: 29 - DNA, 21 bp, Artificial Sequence
  >Homo sapiens
gctttccttggtcaggcagta

SEQ ID NO: 30 - DNA, 21 bp, Artificial Sequence
  >Homo sapiens
acttcgtggggtccttttcac

SEQ ID NO: 31 - DNA, 20 bp, Artificial Sequence
  >Homo sapiens
tctcgcatgaaggagacaca

SEQ ID NO: 32 - DNA, 18 bp, Artificial Sequence
  >Homo sapiens
cgcactcgctccacaaaa

SEQ ID NO: 33 - DNA, 22 bp, Artificial Sequence
  >Homo sapiens
tcttcactgaggtggagatgac

SEQ ID NO: 34 - DNA, 20 bp, Artificial Sequence
  >Homo sapiens
gccagagttgcattcttcca

SEQ ID NO: 35 - DNA, 17 bp, Artificial Sequence
  >Homo sapiens
cggatgcgctgcaggaa

SEQ ID NO: 36 - DNA, 20 bp, Artificial Sequence
  >Homo sapiens
ccaggttgctgttcctctca

SEQ ID NO: 37 - DNA, 20 bp, Artificial Sequence
  >Homo sapiens
atgtacccctccatggatca

SEQ ID NO: 38 - DNA, 20 bp, Artificial Sequence
  >Homo sapiens
ctcctgttcccatgccaata

SEQ ID NO: 39 - DNA, 20 bp, Artificial Sequence
  >Homo sapiens
gcaagaagtgctttgcccta

SEQ ID NO: 40 - DNA, 17 bp, Artificial Sequence
  >Homo sapiens
aaggcggctgccacata

SEQ ID NO: 41 - DNA, 24 bp, Artificial Sequence
  >Homo sapiens
acctgaattagcactggatactcc

SEQ ID NO: 42 - DNA, 22 bp, Artificial Sequence
  >Homo sapiens
ccatctccaacagctctagcaa

SEQ ID NO: 43 - DNA, 21 bp, Artificial Sequence
  >Homo sapiens
gtggaatggcttttaccttcc

SEQ ID NO: 44 - DNA, 20 bp, Artificial Sequence
  >Homo sapiens
cttggctccctcttcatcaa

SEQ ID NO: 45 - DNA, 18 bp, Artificial Sequence
  >Homo sapiens
gcgacctggaagtccaac

SEQ ID NO: 46 - DNA, 20 bp, Artificial Sequence
  >Homo sapiens
cacattgtctgctcccacaa

SEQ ID NO: 47 - DNA, 20 bp, Artificial Sequence
  >Homo sapiens
ggcagctcccaatgtcttac

SEQ ID NO: 48 - DNA, 22 bp, Artificial Sequence
  >Homo sapiens
acatataagtggctcccgtaca

SEQ ID NO: 49 - DNA, 20 bp, Artificial Sequence
  >Homo sapiens
ctggacagccacctcatcaa

SEQ ID NO: 50 - DNA, 22 bp, Artificial Sequence
  >Homo sapiens
tagcggtagtagtcacccttca

SEQ ID NO: 51 - DNA, 19 bp, Artificial Sequence
  >Homo sapiens
atgctggcaccagaacgaa

SEQ ID NO: 52 - DNA, 21 bp, Artificial Sequence
  >Homo sapiens
gctggcacaattgggtttcaa

SEQ ID NO: 53 - DNA, 20 bp, Artificial Sequence
  >Homo sapiens
agcagctcaggaggctgtta

SEQ ID NO: 54 - DNA, 22 bp, Artificial Sequence
  >Homo sapiens
gcaactgagatgcagacaccaa

SEQ ID NO: 55 - DNA, 21 bp, Artificial Sequence
  >Homo sapiens
gcaatgagtttggggagatcc

SEQ ID NO: 56 - DNA, 19 bp, Artificial Sequence
  >Homo sapiens
ctggtcatccacgactcca

SEQ ID NO: 57 - DNA, 19 bp, Artificial Sequence
  >Homo sapiens
catgggacccactcagtca

SEQ ID NO: 58 - DNA, 21 bp, Artificial Sequence
  >Homo sapiens
ccagtatttgagcgtccttcc

SEQ ID NO: 59 - DNA, 21 bp, Artificial Sequence
  >Homo sapiens
cctgtgaagtggatgccctta

SEQ ID NO: 60 - DNA, 21 bp, Artificial Sequence
  >Homo sapiens
caacggcaaagttctcttcca

SEQ ID NO: 61 - DNA, 21 bp, Artificial Sequence
  >Homo sapiens
gcgtggcttttcctcatatca

SEQ ID NO: 62 - DNA, 20 bp, Artificial Sequence
  >Homo sapiens
gtattgccgcaagtcttcca